European Patent Application EP 4 424 325 A1, published September 4, 2024. Title: Human transferrin receptor-affinity peptide. Applicant: JCR Pharmaceuticals Co., Ltd. Application JP. The sequence listing filed with the application follows.

SEQUENCE LISTING (69 sequences)

SEQ ID NO: 1 - protein, 760 aa, Homo sapiens
  REGION 1..760: note = Amino acid sequence of human transferrin receptor
MMDQARSAFSNLFGGEPLSYTRFSLARQVDGDNSHVEMKLAVDEEENADNNTKANVTKPKRCSGSICYGTIAVIVFFLIGFMIGYLGYCKGVEPKTECERLAGTESPVREEPGEDFPAARRLYWDDLKRKLSEKLDSTDFTGTIKLLNENSYVPREAGSQKDENLALYVENQFREFKLSKVWRDQHFVKIQVKDSAQNSVIIVDKNGRLVYLVENPGGYVAYSKAATVTGKLVHANFGTKKDFEDLYTPVNGSIVIVRAGKITFAEKVANAESLNAIGVLIYMDQTKFPIVNAELSFFGHAHLGTGDPYTPGFPSFNHTQFPPSRSSGLPNIPVQTISRAAAEKLFGNMEGDCPSDWKTDSTCRMVTSESKNVKLTVSNVLKEIKILNIFGVIKGFVEPDHYVVVGAQRDAWGPGAAKSGVGTALLLKLAQMFSDMVLKDGFQPSRSIIFASWSAGDFGSVGATEWLEGYLSSLHLKAFTYINLDKAVLGTSNFKVSASPLLYTLIEKTMQNVKHPVTGQFLYQDSNWASKVEKLTLDNAAFPFLAYSGIPAVSFCFCEDTDYPYLGTTMDTYKELIERIPELNKVARAAAEVAGQFVIKLTHDVELNLDYERYNSQLLSFVRDLNQYRADIKEMGLSLQWLYSARGDFFRATSRLTTDFGNAEKTDRFVMKKLNDRVMRVEYHFLSPYVSPKESPFRHVFWGSGSHTLPALLENLKLRKQNNGAFNETLFRNQLALATWTIQGAANALSGDVWDIDNEF

SEQ ID NO: 2 - protein, 760 aa, Macaca fascicularis
  REGION 1..760: note = Amino acid sequence of monkey transferrin receptor
MMDQARSAFSNLFGGEPLSYTRFSLARQVDGDNSHVEMKLAVDDEENADNNTKANGTKPKRCGGNICYGTIAVIIFFLIGFMIGYLGYCKGVEPKTECERLAGTESPAREEPEEDFPAAPRLYWDDLKRKLSEKLDTTDFTSTIKLLNENLYVPREAGSQKDENLALYIENQFREFKLSKVWRDQHFVKIQVKDSAQNSVIIVDKNGGLVYLVENPGGYVAYSKAATVTGKLVHANFGTKKDFEDLDSPVNGSIVIVRAGKITFAEKVANAESLNAIGVLIYMDQTKFPIVKADLSFFGHAHLGTGDPYTPGFPSFNHTQFPPSQSSGLPNIPVQTISRAAAEKLFGNMEGDCPSDWKTDSTCKMVTSENKSVKLTVSNVLKETKILNIFGVIKGFVEPDHYVVVGAQRDAWGPGAAKSSVGTALLLKLAQMFSDMVLKDGFQPSRSIIFASWSAGDFGSVGATEWLEGYLSSLHLKAFTYINLDKAVLGTSNFKVSASPLLYTLIEKTMQDVKHPVTGRSLYQDSNWASKVEKLTLDNAAFPFLAYSGIPAVSFCFCEDTDYPYLGTTMDTYKELVERIPELNKVARAAAEVAGQFVIKLTHDTELNLDYERYNSQLLLFLRDLNQYRADVKEMGLSLQWLYSARGDFFRATSRLTTDFRNAEKRDKFVMKKLNDRVMRVEYYFLSPYVSPKESPFRHVFWGSGSHTLSALLESLKLRRQNNSAFNETLFRNQLALATWTIQGAANALSGDVWDIDNEF

SEQ ID NO: 3 - protein, 113 aa, synthetic construct
  REGION 1..113: note = Amino acid sequence of hTfR-affinity peptide 1
QVQLVESGGGLVHPGGSLRLSCVASGTSFSLNVVTWYRQALGKQREWVATINQSEAPTYADSVKGRFTISRDGAKNTVYLQMNSLVTEDTALYYCYDRYNEIRGQGTQVTVSS

SEQ ID NO: 4 - protein, 113 aa, synthetic construct
  REGION 1..113: note = Amino acid sequence of hTfR-affinity peptide 2
QVQLVESGGGLVHPGGSLSLSCAASGTSFSFNTVTWYRQALGKQREWVATINGSGAPTYADSVKGRFTISRDGAKNTVYLLMNSLVTEDTALYYCYDRYNEIRGQGTQVTVSS

SEQ ID NO: 5 - protein, 116 aa, synthetic construct
  REGION 1..116: note = Amino acid sequence of hTfR-affinity peptide 3
QVQLVESGGGLVQPGESLRLSCAASGSIFDIYVMRWYRQAPGNQREWVASIYDGGRNDYDNVVKGRFTISRDNAKNTVHLQMNSLKPEDTAVYFCNVLTYAGRPYWGQGTQVTVSS

SEQ ID NO: 6 - protein, 120 aa, synthetic construct
  REGION 1..120: note = Amino acid sequence of hTfR-affinity peptide 4
QVQLVESGGGLVQAGASLRLSCAASGRTDGIDRMAWFHQAPGEGREFVAGINKRGGGVDYAPGVKGRFTLSLDSDKNTLYLQMNNLRLEDTGVYSCAVGSGRIIVKSDTWGQGTQVTVSS

SEQ ID NO: 7 - protein, 116 aa, synthetic construct
  REGION 1..116: note = Amino acid sequence of hTfR-affinity peptide 5
QVQLVESGGGLVQPGGSLRLSCAASGSIFDIYVMRWYRQAPGKGLEWVASIYDGGRNDYDNVVKGRFTISRDNSKNTLYLQMNSLRAEDTAVYFCNVLTYAGRPYWGQGTQVTVSS

SEQ ID NO: 8 - protein, 9 aa, synthetic construct
  REGION 1..9: note = Amino acid sequence of CDR1 of hTfR-affinity peptide 1 (1)
GTSFSLNVV

SEQ ID NO: 9 - protein, 10 aa, synthetic construct
  REGION 1..10: note = Amino acid sequence of CDR1 of hTfR-affinity peptide 1 (2)
GTSFSLNVVT

SEQ ID NO: 10 - protein, 9 aa, synthetic construct
  REGION 1..9: note = Amino acid sequence of CDR2 of hTfR-affinity peptide 1 (1)
TINQSEAPT

SEQ ID NO: 11 - protein, 13 aa, synthetic construct
  REGION 1..13: note = Amino acid sequence of CDR2 of hTfR-affinity peptide 1 (2)
TINQSEAPTYADS

SEQ ID NO: 12 - protein, 6 aa, synthetic construct
  REGION 1..6: note = Amino acid sequence of CDR3 of hTfR-affinity peptide 1 (1)
RYNEIR

SEQ ID NO: 13 - protein, 8 aa, synthetic construct
  REGION 1..8: note = Amino acid sequence of CDR3 of hTfR-affinity peptide 1 (2)
YDRYNEIR

SEQ ID NO: 14 - protein, 9 aa, synthetic construct
  REGION 1..9: note = Amino acid sequence of CDR1 of hTfR-affinity peptide 2 (1)
GTSFSFNTV

SEQ ID NO: 15 - protein, 10 aa, synthetic construct
  REGION 1..10: note = Amino acid sequence of CDR1 of hTfR-affinity peptide 2 (2)
GTSFSFNTVT

SEQ ID NO: 16 - protein, 8 aa, synthetic construct
  REGION 1..8: note = Amino acid sequence of CDR2 of hTfR-affinity peptide 2 (1)
INGSGAPT

SEQ ID NO: 17 - protein, 12 aa, synthetic construct
  REGION 1..12: note = Amino acid sequence of CDR2 of hTfR-affinity peptide 2 (2)
INGSGAPTYADS

SEQ ID NO: 18 - protein, 6 aa, synthetic construct
  REGION 1..6: note = Amino acid sequence of CDR3 of hTfR-affinity peptide 2 (1)
RYNEIR

SEQ ID NO: 19 - protein, 8 aa, synthetic construct
  REGION 1..8: note = Amino acid sequence of CDR3 of hTfR-affinity peptide 2 (2)
YDRYNEIR

SEQ ID NO: 20 - protein, 9 aa, synthetic construct
  REGION 1..9: note = Amino acid sequence of CDR1 of hTfR-affinity peptide 3 (1)
GSIFDIYVM

SEQ ID NO: 21 - protein, 10 aa, synthetic construct
  REGION 1..10: note = Amino acid sequence of CDR1 of hTfR-affinity peptide 3 (2)
GSIFDIYVMR

SEQ ID NO: 22 - protein, 8 aa, synthetic construct
  REGION 1..8: note = Amino acid sequence of CDR2 of hTfR-affinity peptide 3 (1)
IYDGGRND

SEQ ID NO: 23 - protein, 12 aa, synthetic construct
  REGION 1..12: note = Amino acid sequence of CDR2 of hTfR-affinity peptide 3 (2)
IYDGGRNDYDNV

SEQ ID NO: 24 - protein, 8 aa, synthetic construct
  REGION 1..8: note = Amino acid sequence of CDR3 of hTfR-affinity peptide 3 (1)
LTYAGRPY

SEQ ID NO: 25 - protein, 11 aa, synthetic construct
  REGION 1..11: note = Amino acid sequence of CDR3 of hTfR-affinity peptide 3 (2)
NVLTYAGRPYW

SEQ ID NO: 26 - protein, 9 aa, synthetic construct
  REGION 1..9: note = Amino acid sequence of CDR1 of hTfR-affinity peptide 4 (1)
GRTDGIDRM

SEQ ID NO: 27 - protein, 10 aa, synthetic construct
  REGION 1..10: note = Amino acid sequence of CDR1 of hTfR-affinity peptide 4 (2)
GRTDGIDRMA

SEQ ID NO: 28 - protein, 9 aa, synthetic construct
  REGION 1..9: note = Amino acid sequence of CDR2 of hTfR-affinity peptide 4 (1)
INKRGGGVD

SEQ ID NO: 29 - protein, 13 aa, synthetic construct
  REGION 1..13: note = Amino acid sequence of CDR2 of hTfR-affinity peptide 4 (2)
INKRGGGVDYAPG

SEQ ID NO: 30 - protein, 11 aa, synthetic construct
  REGION 1..11: note = Amino acid sequence of CDR3 of hTfR-affinity peptide 4 (1)
GSGRIIVKSDT

SEQ ID NO: 31 - protein, 14 aa, synthetic construct
  REGION 1..14: note = Amino acid sequence of CDR3 of hTfR-affinity peptide 4 (2)
AVGSGRIIVKSDTW

SEQ ID NO: 32 - protein, 5 aa, synthetic construct
  REGION 1..5: note = Amino acid sequence of an exemplified linker 1
GGGGS

SEQ ID NO: 33 - protein, 6 aa, synthetic construct
  REGION 1..6: note = Amino acid sequence of an exemplified linker 2
GGGGGS

SEQ ID NO: 34 - protein, 5 aa, synthetic construct
  REGION 1..5: note = Amino acid sequence of an exemplified linker 3
SGGGG

SEQ ID NO: 35 - protein, 33 aa, synthetic construct
  REGION 1..33: note = Amino acid sequence of an exemplified linker 4
GGGGGSGGGGGSGGGGGSGGGGGSGGGGGSGGS

SEQ ID NO: 36 - protein, 32 aa, synthetic construct
  REGION 1..32: note = Amino acid sequence of an exemplified linker 5
GGGGGSGGGGGSGGGGGSGGGGGSGGGGGSGS

SEQ ID NO: 37 - protein, 218 aa, Homo sapiens
  REGION 1..218: note = Amino acid sequence of an exemplified Fc region of human IgG
PAPELLGGPSVFLFPPKPKDTLMISRTPEVTCVVVDVSHEDPEVKFNWYVDGVEVHNAKTKPREEQYNSTYRVVSVLTVLHQDWLNGKEYKCKVSNKALPAPIEKTISKAKGQPREPQVYTLPPSREEMTKNQVSLTCLVKGFYPSDIAVEWESNGQPENNYKTTPPVLDSDGSFFLYSKLTVDKSRWQQGNVFSCSVMHEALHNHYTQKSLSLSPGK

SEQ ID NO: 38 - protein, 585 aa, Homo sapiens [sequence omitted]

SEQ ID NO: 39 - protein, 46 aa, Streptococcus sp. G148
  REGION 1..46: note = Amino acid sequence of albumin binding domain
LAEAKVLALRELDKYGVSDYYKDLIDKAKTVEGVKALIDEILAALP

SEQ ID NO: 40 - protein, 451 aa, synthetic construct
  REGION 1..451: note = Amino acid sequence of heavy chain of Trastuzumab
EVQLVESGGGLVQPGGSLRLSCAASGFNIKDTYIHWVRQAPGKGLEWVARIYPTNGYTRYADSVKGRFTISADTSKNTAYLQMNSLRAEDTAVYYCSRWGGDGFYAMDYWGQGTLVTVSSASTKGPSVFPLAPSSKSTSGGTAALGCLVKDYFPEPVTVSWNSGALTSGVHTFPAVLQSSGLYSLSSVVTVPSSSLGTQTYICNVNHKPSNTKVDKKVEPPKSCDKTHTCPPCPAPELLGGPSVFLFPPKPKDTLMISRTPEVTCVVVDVSHEDPEVKFNWYVDGVEVHNAKTKPREEQYNSTYRVVSVLTVLHQDWLNGKEYKCKVSNKALPAPIEKTISKAKGQPREPQVYTLPPSRDELTKNQVSLTCLVKGFYPSDIAVEWESNGQPENNYKTTPPVLDSDGSFFLYSKLTVDKSRWQQGNVFSCSVMHEALHNHYTQKSLSLSPGK

SEQ ID NO: 41 - protein, 214 aa, synthetic construct
  REGION 1..214: note = Amino acid sequence of light chain of Trastuzumab
DIQMTQSPSSLSASVGDRVTITCRASQDVNTAVAWYQQKPGKAPKLLIYSASFLYSGVPSRFSGSRSGTDFTLTISSLQPEDFATYYCQQHYTTPPTFGQGTKVEIKRTVAAPSVFIFPPSDEQLKSGTASVVCLLNNFYPREAKVQWKVDNALQSGNSQESVTEQDSKDSTYSLSSTLTLSKADYEKHKVYACEVTHQGLSSPVTKSFNRGEC

SEQ ID NO: 42 - protein, 611 aa, synthetic construct
  REGION 1..611: note = Amino acid sequence of the fusion protein of hTfR-affinitypeptide 1 and heavy chain of Trastuzumab
MGWSCIILFLVATATGVHSEVQLVESGGGLVQPGGSLRLSCAASGFNIKDTYIHWVRQAPGKGLEWVARIYPTNGYTRYADSVKGRFTISADTSKNTAYLQMNSLRAEDTAVYYCSRWGGDGFYAMDYWGQGTLVTVSSASTKGPSVFPLAPSSKSTSGGTAALGCLVKDYFPEPVTVSWNSGALTSGVHTFPAVLQSSGLYSLSSVVTVPSSSLGTQTYICNVNHKPSNTKVDKKVEPPKSCDKTHTCPPCPAPELLGGPSVFLFPPKPKDTLMISRTPEVTCVVVDVSHEDPEVKFNWYVDGVEVHNAKTKPREEQYNSTYRVVSVLTVLHQDWLNGKEYKCKVSNKALPAPIEKTISKAKGQPREPQVYTLPPSRDELTKNQVSLTCLVKGFYPSDIAVEWESNGQPENNYKTTPPVLDSDGSFFLYSKLTVDKSRWQQGNVFSCSVMHEALHNHYTQKSLSLSPGKGGGGSGGGGSGGGGSGGGGSGGGGSGGSQVQLVESGGGLVHPGGSLRLSCVASGTSFSLNVVTWYRQALGKQREWVATINQSEAPTYADSVKGRFTISRDGAKNTVYLQMNSLVTEDTALYYCYDRYNEIRGQGTQVTVSS

SEQ ID NO: 43 - protein, 611 aa, synthetic construct
  REGION 1..611: note = Amino acid sequence of the fusion protein of hTfR-affinitypeptide 2 and heavy chain of Trastuzumab
MGWSCIILFLVATATGVHSEVQLVESGGGLVQPGGSLRLSCAASGFNIKDTYIHWVRQAPGKGLEWVARIYPTNGYTRYADSVKGRFTISADTSKNTAYLQMNSLRAEDTAVYYCSRWGGDGFYAMDYWGQGTLVTVSSASTKGPSVFPLAPSSKSTSGGTAALGCLVKDYFPEPVTVSWNSGALTSGVHTFPAVLQSSGLYSLSSVVTVPSSSLGTQTYICNVNHKPSNTKVDKKVEPPKSCDKTHTCPPCPAPELLGGPSVFLFPPKPKDTLMISRTPEVTCVVVDVSHEDPEVKFNWYVDGVEVHNAKTKPREEQYNSTYRVVSVLTVLHQDWLNGKEYKCKVSNKALPAPIEKTISKAKGQPREPQVYTLPPSRDELTKNQVSLTCLVKGFYPSDIAVEWESNGQPENNYKTTPPVLDSDGSFFLYSKLTVDKSRWQQGNVFSCSVMHEALHNHYTQKSLSLSPGKGGGGSGGGGSGGGGSGGGGSGGGGSGGSQVQLVESGGGLVHPGGSLSLSCAASGTSFSFNTVTWYRQALGKQREWVATINGSGAPTYADSVKGRFTISRDGAKNTVYLLMNSLVTEDTALYYCYDRYNEIRGQGTQVTVSS

SEQ ID NO: 44 - protein, 614 aa, synthetic construct
  REGION 1..614: note = Amino acid sequence of the fusion protein of hTfR-affinitypeptide 3 and heavy chain of Trastuzumab
MGWSCIILFLVATATGVHSEVQLVESGGGLVQPGGSLRLSCAASGFNIKDTYIHWVRQAPGKGLEWVARIYPTNGYTRYADSVKGRFTISADTSKNTAYLQMNSLRAEDTAVYYCSRWGGDGFYAMDYWGQGTLVTVSSASTKGPSVFPLAPSSKSTSGGTAALGCLVKDYFPEPVTVSWNSGALTSGVHTFPAVLQSSGLYSLSSVVTVPSSSLGTQTYICNVNHKPSNTKVDKKVEPPKSCDKTHTCPPCPAPELLGGPSVFLFPPKPKDTLMISRTPEVTCVVVDVSHEDPEVKFNWYVDGVEVHNAKTKPREEQYNSTYRVVSVLTVLHQDWLNGKEYKCKVSNKALPAPIEKTISKAKGQPREPQVYTLPPSRDELTKNQVSLTCLVKGFYPSDIAVEWESNGQPENNYKTTPPVLDSDGSFFLYSKLTVDKSRWQQGNVFSCSVMHEALHNHYTQKSLSLSPGKGGGGSGGGGSGGGGSGGGGSGGGGSGGSQVQLVESGGGLVQPGESLRLSCAASGSIFDIYVMRWYRQAPGNQREWVASIYDGGRNDYDNVVKGRFTISRDNAKNTVHLQMNSLKPEDTAVYFCNVLTYAGRPYWGQGTQVTVSS

SEQ ID NO: 45 - protein, 618 aa, synthetic construct
  REGION 1..618: note = Amino acid sequence of the fusion protein of hTfR-affinitypeptide 4 and heavy chain of Trastuzumab
MGWSCIILFLVATATGVHSEVQLVESGGGLVQPGGSLRLSCAASGFNIKDTYIHWVRQAPGKGLEWVARIYPTNGYTRYADSVKGRFTISADTSKNTAYLQMNSLRAEDTAVYYCSRWGGDGFYAMDYWGQGTLVTVSSASTKGPSVFPLAPSSKSTSGGTAALGCLVKDYFPEPVTVSWNSGALTSGVHTFPAVLQSSGLYSLSSVVTVPSSSLGTQTYICNVNHKPSNTKVDKKVEPPKSCDKTHTCPPCPAPELLGGPSVFLFPPKPKDTLMISRTPEVTCVVVDVSHEDPEVKFNWYVDGVEVHNAKTKPREEQYNSTYRVVSVLTVLHQDWLNGKEYKCKVSNKALPAPIEKTISKAKGQPREPQVYTLPPSRDELTKNQVSLTCLVKGFYPSDIAVEWESNGQPENNYKTTPPVLDSDGSFFLYSKLTVDKSRWQQGNVFSCSVMHEALHNHYTQKSLSLSPGKGGGGSGGGGSGGGGSGGGGSGGGGSGGSQVQLVESGGGLVQAGASLRLSCAASGRTDGIDRMAWFHQAPGEGREFVAGINKRGGGVDYAPGVKGRFTLSLDSDKNTLYLQMNNLRLEDTGVYSCAVGSGRIIVKSDTWGQGTQVTVSS

SEQ ID NO: 46 - protein, 614 aa, synthetic construct
  REGION 1..614: note = Amino acid sequence of the fusion protein of hTfR-affinitypeptide 5 and heavy chain of Trastuzumab
MGWSCIILFLVATATGVHSEVQLVESGGGLVQPGGSLRLSCAASGFNIKDTYIHWVRQAPGKGLEWVARIYPTNGYTRYADSVKGRFTISADTSKNTAYLQMNSLRAEDTAVYYCSRWGGDGFYAMDYWGQGTLVTVSSASTKGPSVFPLAPSSKSTSGGTAALGCLVKDYFPEPVTVSWNSGALTSGVHTFPAVLQSSGLYSLSSVVTVPSSSLGTQTYICNVNHKPSNTKVDKKVEPPKSCDKTHTCPPCPAPELLGGPSVFLFPPKPKDTLMISRTPEVTCVVVDVSHEDPEVKFNWYVDGVEVHNAKTKPREEQYNSTYRVVSVLTVLHQDWLNGKEYKCKVSNKALPAPIEKTISKAKGQPREPQVYTLPPSRDELTKNQVSLTCLVKGFYPSDIAVEWESNGQPENNYKTTPPVLDSDGSFFLYSKLTVDKSRWQQGNVFSCSVMHEALHNHYTQKSLSLSPGKGGGGSGGGGSGGGGSGGGGSGGGGSGGSQVQLVESGGGLVQPGGSLRLSCAASGSIFDIYVMRWYRQAPGKGLEWVASIYDGGRNDYDNVVKGRFTISRDNSKNTLYLQMNSLRAEDTAVYFCNVLTYAGRPYWGQGTQVTVSS

SEQ ID NO: 47 - DNA, 1836 bp, synthetic construct
  misc_feature 1..1836: note = Nucleotide sequence of the DNA encoding the fusion protein ofhTfR-affinity peptide 1 and heavy chain of Trastuzumab, syntheticsequence
  source 1..1836: mol_type = other DNA
atgggctggagctgcattattctgtttctggtggcgaccgcgaccggcgtgcatagcgaagtgcagctggtggaaagcggcggcggcctggtgcagccgggcggcagcctgcgcctgagctgcgcggcgagcggctttaacattaaagatacctatattcattgggtgcgccaggcgccgggcaaaggcctggaatgggtggcgcgcatttatccgaccaacggctatacccgctatgcggatagcgtgaaaggccgctttaccattagcgcggataccagcaaaaacaccgcgtatctgcagatgaacagcctgcgcgcggaagataccgcggtgtattattgcagccgctggggcggcgatggcttttatgcgatggattattggggccagggcaccctggtgaccgtgagcagcgcgagcaccaaaggcccgagcgtgtttccgctggcgccgagcagcaaaagcaccagcggcggcaccgcggcgctgggctgcctggtgaaagattattttccggaaccggtgaccgtgagctggaacagcggcgcgctgaccagcggcgtgcatacctttccggcggtgctgcagagcagcggcctgtatagcctgagcagcgtggtgaccgtgccgagcagcagcctgggcacccagacctatatttgcaacgtgaaccataaaccgagcaacaccaaagtggataaaaaagtggaaccgccgaaaagctgcgataaaacccatacctgcccgccgtgcccggcgccggaactgctgggcggcccgagcgtgtttctgtttccgccgaaaccgaaagataccctgatgattagccgcaccccggaagtgacctgcgtggtggtggatgtgagccatgaagatccggaagtgaaatttaactggtatgtggatggcgtggaagtgcataacgcgaaaaccaaaccgcgcgaagaacagtataacagcacctatcgcgtggtgagcgtgctgaccgtgctgcatcaggattggctgaacggcaaagaatataaatgcaaagtgagcaacaaagcgctgccggcgccgattgaaaaaaccattagcaaagcgaaaggccagccgcgcgaaccgcaggtgtataccctgccgccgagccgcgatgaactgaccaaaaaccaggtgagcctgacctgcctggtgaaaggcttttatccgagcgatattgcggtggaatgggaaagcaacggccagccggaaaacaactataaaaccaccccgccggtgctggatagcgatggcagcttttttctgtatagcaaactgaccgtggataaaagccgctggcagcagggcaacgtgtttagctgcagcgtgatgcatgaagcgctgcataaccattatacccagaaaagcctgagcctgagcccgggcaaaggtggcggagggtctggaggtggcggatcaggcggaggaggttccgggggcggtggaagcggaggcggtggaagtggcggatcccaggtgcagctcgtggagtctgggggaggcttggtgcaccctggggggtctctgagactctcctgtgtagcctcaggaacctccttcagtctcaatgtcgtgacctggtaccgccaggctctagggaagcagcgcgagtgggtcgcaactattaatcagagcgaggcccctacctatgcagactccgtgaagggccgatttaccatctccagagacggcgccaagaacacggtgtatctgcaaatgaacagcctagtgactgaggatacggccctctattactgttatgaccggtacaacgaaatccggggccaggggacccaggtcaccgtctcctcataa

SEQ ID NO: 48 - DNA, 702 bp, synthetic construct
  misc_feature 1..702: note = Nucleotide sequence of the DNA encoding the light chain ofTrastuzumab, synthetic sequence
  source 1..702: mol_type = other DNA
atgggctggagctgcattattctgtttctggtggcgaccgcgaccggcgtgcatagcgatattcagatgacccagagcccgagcagcctgagcgcgagcgtgggcgatcgcgtgaccattacctgccgcgcgagccaggatgtgaacaccgcggtggcgtggtatcagcagaaaccgggcaaagcgccgaaactgctgatttatagcgcgagctttctgtatagcggcgtgccgagccgctttagcggcagccgcagcggcaccgattttaccctgaccattagcagcctgcagccggaagattttgcgacctattattgccagcagcattataccaccccgccgacctttggccagggcaccaaagtggaaattaaacgcaccgtggcggcgccgagcgtgtttatttttccgccgagcgatgaacagctgaaaagcggcaccgcgagcgtggtgtgcctgctgaacaacttttatccgcgcgaagcgaaagtgcagtggaaagtggataacgcgctgcagagcggcaacagccaggaaagcgtgaccgaacaggatagcaaagatagcacctatagcctgagcagcaccctgaccctgagcaaagcggattatgaaaaacataaagtgtatgcgtgcgaagtgacccatcagggcctgagcagcccggtgaccaaaagctttaaccgcggcgaatgctaa

SEQ ID NO: 49 - DNA, 43 bp, synthetic construct
  misc_feature 1..43: note = Primer hTfR5', synthetic sequence
  source 1..43: mol_type = other DNA
ccgacgcgtcgccaccatgatggatcaagctagatcagcattc

SEQ ID NO: 50 - DNA, 59 bp, synthetic construct
  misc_feature 1..59: note = Primer hTfR3', synthetic sequence
  source 1..59: mol_type = other DNA
ataatgcggccgcttaatgatgatgatgatgatgaaactcattgtcaatgtcccaaacg

SEQ ID NO: 51 - DNA, 4460 bp, synthetic construct
  misc_feature 1..4460: note = Nucleotide sequence of the DNA formed of a cDNA encodingchimerichTfR and a loxP-flanked neomycin resistance gene placedon the cDNA's 3' side, synthetic sequence
  source 1..4460: mol_type = other DNA
gtttatcctcccttgtagcagctgagaatgatggatcaagccagatcagcattctctaacttgtttggtggggaaccattgtcatacacccggtttagccttgctcggcaagtagatggagataacagtcatgtggagatgaaactggctgcagatgaagaagaaaatgccgacaataacatgaaggctagtgtcagaaaacccaagaggtttaatggaagactctgctttgcagctattgcactagtcattttcttcttgattggattcatgagtggctacctgggctattgtaaaggggtagaaccaaaaactgagtgtgagagactggcaggaaccgagtctccagtgagggaggagccaggagaggacttccctgcagcacgtcgcttatattgggatgacctgaagagaaagttgtcggagaaactggacagcacagacttcaccggcaccatcaagctgctgaatgaaaattcatatgtccctcgtgaggctggatctcaaaaagatgaaaatcttgcgttgtatgttgaaaatcaatttcgtgaatttaaactcagcaaagtctggcgtgatcaacattttgttaagattcaggtcaaagacagcgctcaaaactcggtgatcatagttgataagaacggtagacttgtttacctggtggagaatcctgggggttatgtggcgtatagtaaggctgcaacagttactggtaaactggtccatgctaattttggtactaaaaaagattttgaggatttatacactcctgtgaatggatctatagtgattgtcagagcagggaaaatcacctttgcagaaaaggttgcaaatgctgaaagcttaaatgcaattggtgtgttgatatacatggaccagactaaatttcccattgttaacgcagaactttcattctttggacatgctcatctggggacaggtgacccttacacacctggattcccttccttcaatcacactcagtttccaccatctcggtcatcaggattgcctaatatacctgtccagacaatctccagagctgctgcagaaaagctgtttgggaatatggaaggagactgtccctctgactggaaaacagactctacatgtaggatggtaacctcagaaagcaagaatgtgaagctcactgtgagcaatgtgctgaaagagataaaaattcttaacatctttggagttattaaaggctttgtagaaccagatcactatgttgtagttggggcccagagagatgcatggggccctggagctgcaaaatccggtgtaggcacagctctcctattgaaacttgcccagatgttctcagatatggtcttaaaagatgggtttcagcccagcagaagcattatctttgccagttggagtgctggagactttggatcggttggtgccactgaatggctagagggatacctttcgtccctgcatttaaaggctttcacttatattaatctggataaagcggttcttggtaccagcaacttcaaggtttctgccagcccactgttgtatacgcttattgagaaaacaatgcaaaatgtgaagcatccggttactgggcaatttctatatcaggacagcaactgggccagcaaagttgagaaactcactttagacaatgctgctttccctttccttgcatattctggaatcccagcagtttctttctgtttttgcgaggacacagattatccttatttgggtaccaccatggacacctataaggaactgattgagaggattcctgagttgaacaaagtggcacgagcagctgcagaggtcgctggtcagttcgtgattaaactaacccatgatgttgaattgaacctggactatgagaggtacaacagccaactgctttcatttgtgagggatctgaaccaatacagagcagacataaaggaaatgggcctgagtttacagtggctgtattctgctcgtggagacttcttccgtgctacttccagactaacaacagatttcgggaatgctgagaaaacagacagatttgtcatgaagaaactcaatgatcgtgtcatgagagtggagtatcacttcctctctccctacgtatctccaaaagagtctcctttccgacatgtcttctggggctccggctctcacacgctgccagctttactggagaacttgaaactgcgtaaacaaaataacggtgcttttaatgaaacgctgttcagaaaccagttggctctagctacttggactattcagggagctgcaaatgccctctctggtgacgtttgggacattgacaatgagttttaacgtggctcgctgatcagcctcgactgtgccttctagttgccagccatctgttgtttgcccctcccccgtgccttccttgaccctggaaggtgccactcccactgtcctttcctaataaaatgaggaaattgcatcgcattgtctgagtaggtgtcattctattctggggggtggggtggggcaggacagcaagggggaggattgggaagacaatagcaggcatgctggggatgcggtgggctctatggcttctgaggcggaaagaaccagctggggctcgatcctctagttaagcttcccagcggccgctatcgaattccgatcatattcaataacccttaatataacttcgtataatgtatgctatacgaagttattaggtctgaagaggagtttacgtccagccaagctaattctaccgggtaggggaggcgcttttcccaaggcagtctggagcatgcgctttagcagccccgctgggcacttggcgctacacaagtggcctctggcctcgcacacattccacatccaccggtaggcgccaaccggctccgttctttggtggccccttcgcgccaccttctactcctcccctagtcaggaagttcccccccgccccgcagctcgcgtcgtgcaggacgtgacaaatggaagtagcacgtctcactagtctcgtgcagatggacagcaccgctgagcaatggaagcgggtaggcctttggggcagcggccaatagcagctttgctccttcgctttctgggctcagaggctgggaaggggtgggtccgggggcgggctcaggggcgggctcaggggcggggcgggcgcccgaaggtcctccggaggcccggcattctgcacgcttcaaaagcgcacgtctgccgcgctgttctcctcttcctcatctccgggcctttcgacctgcagccaatatgggatcggccattgaacaagatggattgcacgcaggttctccggccgcttgggtggagaggctattcggctatgactgggcacaacagacaatcggctgctctgatgccgccgtgttccggctgtcagcgcaggggcgcccggttctttttgtcaagaccgacctgtccggtgccctgaatgaactgcaggacgaggcagcgcggctatcgtggctggccacgacgggcgttccttgcgcagctgtgctcgacgttgtcactgaagcgggaagggactggctgctattgggcgaagtgccggggcaggatctcctgtcatctcaccttgctcctgccgagaaagtatccatcatggctgatgcaatgcggcggctgcatacgcttgatccggctacctgcccattcgaccaccaagcgaaacatcgcatcgagcgagcacgtactcggatggaagccggtcttgtcgatcaggatgatctggacgaagagcatcaggggctcgcgccagccgaactgttcgccaggctcaaggcgcgcatgcccgacggcgaggatctcgtcgtgacccatggcgatgcctgcttgccgaatatcatggtggaaaatggccgcttttctggattcatcgactgtggccggctgggtgtggcggaccgctatcaggacatagcgttggctacccgtgatattgctgaagagcttggcggcgaatgggctgaccgcttcctcgtgctttacggtatcgccgctcccgattcgcagcgcatcgccttctatcgccttcttgacgagttcttctgaggggatccgctgtaagtctgcagaaattgatgatctattaaacaataaagatgtccactaaaatggaagtttttcctgtcatactttgttaagaagggtgagaacagagtacctacattttgaatggaaggattggagctacgggggtgggggtggggtgggattagataaatgcctgctctttactgaaggctctttactattgctttatgataatgtttcatagttggatatcataatttaaacaagcaaaaccaaattaagggccagctcattcctcccactcatgatctatagatccctcgatcgagatccggaacccttaatataacttcgtataatgtatgctatacgaagttattaggtccctcgaagaggttcactagttctagagcatttaaatacgtgctagc

SEQ ID NO: 52 - DNA, 5003 bp, synthetic construct
  misc_feature 1..5003: note = Nucleotide sequence of the 5'-arm of targeting vector
  source 1..5003: mol_type = other DNA
aaagacattcccagggtccctaagggctccatctgggagcgcgctatctgtagtcctgttgtggtttaagataccactctctttgttatttgtaaatttaccacaggctgggcagtaaagtacagataggaagaaaagagtgtgaacgtttgcagttttaacagaactccttttatttgctatgcattgcaacaaccctctaaaagcaataatggcgataaacatgcaagttaatctacaactttatcaccctagtaaatcattggttcctatttcccttccataggctgaacatagtgagcactggtagctctttgcttggcttaagcgctgcttgttaaaatctaaaaaaaaaaaaaaaaaagatttgcagttttgctttaaagtttttcctttaaagcatctctgagctgcaaaaactcgtctttaggatatggttttggcggagacctaagcctgcaagtaggaatattttaaagagtaaaggctgatactttcgaacttgcaccgcagggttgggtgtcggtcaaggttaggcggagggcgacaggccaactccaaagacacggcgggggaggggtgcggtggagaaagcgagccgcagccaatcgcacgcgctctcccgacacctgccgccttggcgccttttctaggctactccgcgcacgcactggctgcgcgcgcagttcgcctccagcggtcttgggggagcacctcggtaggtgtacgtgcggaaggaagtgacgtagatccagagggccggccggggggtggggccgagctataagctttgggtgggaggcagcgctgccttcagaaggcgtgcggagcgcgggctgctgcattgcggactgtagaggcgcttcctagtgagtgactcccttgtcagcggcacggcccatcgtggtcctcgcgtggcgggcggaccagagcgagacgccagggcctgggtggtgcgggcggggaggcggaggggtgtcgcggagtccggggctgaggagcgcgggttgcaggtgcagcgcggtgggtgtggggagccgctgtaccctgcgcccctcgggtcctccgggccttcgcaggccagtgctaggccgcgggttcgagagtcaccacgctgaggcgcaggcttgttccgccgggagcacgtggtggcggctggaggaagtcgccccagggaacggctgtcggggtacgtgggtgaccttggggcccctcgcaggagggcgtcacagctgaaaaggacaaagctgttttctattcggttactagtgtcacggacatttagaggggcggggggagcttccaataactgcacgttggaacttcggcaccacctggtcggtttttttgccagtctctccctcttggcccagcgtgtggaatctcatttttctagggcagaataggtctgaacgctgcaggtaatactaagaacgtctctagcatctcctaagatgggagaacgtagaaatacgacctctttgtacgagctcttttagaactagctgtagagaaccagcgtgcaccctggtgttggacagctctctaaaatggtgtttgagggtaagaaaactgcatttgcaaatttttcagttagcacactttgtcccgagcgtaaaatgaaatgatctccttatacttaggcagaagactggactggattgctgttcagtttctgtgctatttttttaaaataggatttaagtgggaaatagttgtgttacagaaattctcggctattctgtgctatttttttttaaataggatttaagtgggaaatagttgtgttacagaaattctcggctacctgatacttttattctaagattagatgagttggctctgagctgtgaaatatgacctctttgacaaagacatttaagctgattcaggatgttatctacaaagaaaacgggatttagcttgtgtgggtccacttgcatttattttctgttaaggattataataaactgctttatacaggaatccaatatcagctgttttttatatagagagcataatactttttactttgagagaggatgttgtcaaggaatggtggctgtgaacctggcctgtgttgactggttagatctgtctgcctaaccccaccctaaggctaagtagttatatgcttgtggcaatgtgcttatttataatagggcaagattatgggctaaatttgggttagacaacaatgaaagttaattaaacgaccctcaggccttgggtctactatgtgtaagtgatttccttctctcccagatgagtgctatacaaaataaacttcagtgacctcaagtggttttgaccttttggttgctattcagaaaactatggaaatgaaaacctgctacctatttcctattgccttttcaatttcccaaagaaggtctcccctatgaatccatgggtagccttgaactcagatccacctgcttctgtttggagagtgataagattaaaggcaagtgccaccacacccagcaaagtaggctcttaaaactaaaacctttgcagtcgggcatggtgccacacacctttggtcccagcactggggggtaaggcagaggcaggtggatcactgagtttgaggtcagctagtgctgaagagtaagagcctgtctttaaaacatctcaacagctgggcagtcgtggtccattcctttaatcccagcacttgggaggcagaggcaagtggatttttgagttcgaggccagcctggtctacagagtgagttccaggacagccagggatacacagagaaaccctgtctcaaaaaaccaaaatataaataaataaataaagattgggagagaagtcaaggatctcataggtggtcagggagctacaactgcagtagtaaagaagtaggacttaaaagaacagggccggcactaattttgaggatctagatcgggccctcaattaaggaacttccttttgtgtgaactcagaatttgaaatgaaatgtgcttgtcagaaccattgcatggcttattttttaatgaaaagtctggctagtatctgcttatcttccagcttccagctcaaagttaaggtcatagatcaaaagaactatgtctttatcttagttgtatcttaatttttattagaattgaatggttttcctaatgtttggtaacatcaaaggtgtgtaagtaaaagtgagaaatcaagattaactttctcttggcaaagattgttgacattggtgacatcttggaccaaatgagaattgttttacttttaaatgtcccatcaacagctctcagttaggctgttctatctggtttgtcttgccatgcttgcagagtatagatttgacaatttgaaaattcaaaaagctatataaataggtatgttgctatatgtaagattttaaatgagtcagttaagacttaaagaataactgggtttattttatcttgtcaggttatcactgtgtagaccaggttgaccttgaaaacaaattctctgcttcccaagtgctgggattaaaggcgtgtgtcactagctctgacactggctactttggaactactatggtgttcacaaatgcagagttgagtgttgggattaaatggaaatttcatgtctttttttttaactttcccttctacacagggcttctctgtgtagtcctggctgtccttgtagctctagactaggctgaattcaaactcagatccacccacctaagtgctgagattaaaggcatgtgccaccactgcccagttctgaattgttggggttttttttttgttgttattcttaattttagttcgatgaattaaaatcgaaataacttgtttcttagaaaaataaggtgtaattgggttataaagccaaatttagacattaataccaacagcctgtttaggctcaaaattgttcaatcattttattagtattattattaatcatatcaacttgagacctgtttgggaaagcagaatattttagggatagctatttcagacaagcattaatgtgttagctgtttttttccccctagaatatgattaaaattggctcagggtggggccttctagttctggctctagcgattgggtctgtttctggtgaggtggtagtgataaactgtaacagaagggacaagagattgggcttctgagaacatgtatgatctggtatgtgactttaatcattaaagcatggggattcaaaaatactaatgaataggccttagaactagtcctgagtgttttgtaaaataacagtcttaattctcctagtttctggatttttttctttgtctttggatactaagtttaagcatttatttggacagagtggtgcccactagctgttctattctagtacttgggaggcaagaggcagaacgaacatggccagcttggacaacttaagaaaactgaaaggcttgccatcctagtttttcttttgattaaacacacttatattctaactagttttctctatcctttgggttttgttttgttttttatttgttttgtagctctagctggctggcttcggaattgcctgcctcccaagtgctaggattaaaggcatcacagtcactacccaattgatatcatgattcttaattcaacttctaagaacaaattatcacactctgaatctaacatggaatagcattatccatgttcagatatctttgtctcaaggctcaggtttatcctttgtagctttctttttgctatcccacctctattcagcatccagtcaaggatcactgagttggttatcagtaaattaaacattttaattaatgtctaggagacaggttatggtatagttctcagtgctgggaagttgacatggtaggatctcagttcatggccagccagaactttctggtgagatcctggttcaagcactacagagcttttctagaaaagtaactatatttaggagtaagtttgatataatgacaatcccatcgtaagccttcagtaacctgatgcattggtctctgttttaatatcaggta

SEQ ID NO: 53 - DNA, 2604 bp, synthetic construct
  misc_feature 1..2604: note = Nucleotide sequence of the 3'-arm of targeting vector
  source 1..2604: mol_type = other DNA
gcattctctaacttggtaaggtactttcatctatctgaaaaaatgttcagtaaaaaacaaaacaaaaacatgacttcacccagtgagtacaagatgatacccccaattttttttttttttattatatgtatgtacactgtagctgtcttcagacacaccagaagagggcgtcagatctcatcagatggttgtgagccaccatgtggttgctgggacttgaacactggacctttggaaaagcagttgggtactcttacccactgagctatcacaccagccccaataccccaaattttgaccagccttttttttttttttttttttttttttaaatctgaactaatggtattaaggtgaaacagattgcacaaaagaggtactaggtttttctttgaggcaaggtctttctatattgcctcaggttgaccttaaactccaacttcctttttttccccaagtgctggagattgtagacagatatatacaacaccccaaaacaaatatgtttagtttcgattaagattcattatgtggggctagagggatgacttagaggttaagaacactgcctgctcttccagaggtcctgagttcaattcccagcaaccacgtggtggctcacaaccatctgtaatgggatccgatgccctctttctggtgtgtttgaagacagctacagtgtcctcatacataaaaaaaataaacaaacagatcttttaaaaaaaaaggtacagtgtacttatacattatataaatgaatgattctttaaaaaattaattatgggaaatacttatgaagaatagggtagctttggctgttttggaaacgttatataacaaggtagaactaaaatgtatgccagtaatcccagaggaatcattagccagtcagggctagtctgagcaatgtggcaagataaacccatctctttaaaaaaaaaaaaaagtattataaatagaaatgttataggaaacaggaaatagaaaccctcgaaaggctgaatgaaagagtattagtgggctggagagatggttcagcggttaagagcactatctcctgagttcagttcccagtgaccacatggtggctcacagccatctgtaatgagatctgacgccctcttctggggtgtctgaagacagcgacagtgtactcacataaaataaatacataaagactgttagttagccttcatctaccatttacagaactgggcacagaaaggagttcatcagttataaagggtaactttccatatgaatgtttgtcatattattatgcatatagtataatgaccaaactactgtaatgtcttaatatttgtatctcttttctcttttttaaaaatatcagtttggtggggaaccattgtcatacacccggtttagccttgctcggcaagtagatggagataacagtcatgtggagatgaaactggctgcagatgaagaagaaaatgccgacaataacatgaaggctagtgtcagaaaacccaagaggtttaatggaagactctgctttgcagctattgcactagtcattttcttcttgattggtaagaatgagtggccattcagaaggatttcttatgactaactagttcttagactagctagttcttagactagctagttcttgtttcttttggatgaggagatgctttgtactttaaatggcactggggctccctacctgccggcagattaggtcctgcaagatgggaaacgtttacattatggatgttttattagagatatgcaggacatttggaatagtactaagaaaggcttccagtaagacaaggtgtgcacccatgtcttaaacaggtcactgtaaaatatgacttagttgtggtaatttaaattccattaaactcaggttcataattttctattagattctcatagtttaattaaaagttttcagggataagttaaaaatgagttctgtgagtttagctctaaaacttcctgtttttaggattcatgagtggctacctgggctattgtaagcgtgtagaacaaaaagaggagtgtgtgaaactggctgaaacggaggagacagacaagtcagaaaccatggaaacagaggatgttcctacatcatctcgcttatattgggcagacctcaaaacactgttgtcagagaagttgaactccatagagtttgctgacaccatcaagtaagctcaacttcccaagttcagtcctgatggaaacgtttttgttgggggggtagggagacttgaaaggctttcagagggtcctcctgacaatgtggaactatgctgacaggaaattaggacttacctggagagcctcatagcctcctttttcttcagaatcgttttatcagttgtagtttagtgtgggatgtcagattttcttctgttctaatattccttttaaaaattttttaaaattaaaattactttttatgtattatgagtatagcctgcatatatgaatgaatgtgcattactaattacacttatctcctagtgcctacataagccttatagatggttgtgagccagcatgtgggtgctggaatccaaaatggttcttgcaagaccaaatatgttacatcccagagccattaca

SEQ ID NO: 54 - protein, 7 aa, synthetic construct
  REGION 1..7: note = Peptide tag
DYKDDDD

SEQ ID NO: 55 - protein, 116 aa, synthetic construct
  REGION 1..116: note = Amino acid sequence of hTfR-affinity peptide 6
QVQLVESGGGLVQPGGSLRLSCAASGSIFDIYVMRWYRQAPGKGLEWVASIYAGGRNDYDNVVKGRFTISRDNSKNTLYLQMNSLRAEDTAVYFCNVLTYAGRPYWGQGTQVTVSS

SEQ ID NO: 56 - protein, 8 aa, synthetic construct
  REGION 1..8: note = Amino acid sequence of CDR2 of hTfR-affinity peptide 6 (1)
IYAGGRND

SEQ ID NO: 57 - protein, 12 aa, synthetic construct
  REGION 1..12: note = Amino acid sequence of CDR2 of hTfR-affinity peptide 6 (2)
IYAGGRNDYDNV

SEQ ID NO: 58 - protein, 525 aa, Homo sapiens
  REGION 1..525: note = Amino acid sequence of hIDS
SETQANSTTDALNVLLIIVDDLRPSLGCYGDKLVRSPNIDQLASHSLLFQNAFAQQAVCAPSRVSFLTGRRPDTTRLYDFNSYWRVHAGNFSTIPQYFKENGYVTMSVGKVFHPGISSNHTDDSPYSWSFPPYHPSSEKYENTKTCRGPDGELHANLLCPVDVLDVPEGTLPDKQSTEQAIQLLEKMKTSASPFFLAVGYHKPHIPFRYPKEFQKLYPLENITLAPDPEVPDGLPPVAYNPWMDIRQREDVQALNISVPYGPIPVDFQRKIRQSYFASVSYLDTQVGRLLSALDDLQLANSTIIAFTSDHGWALGEHGEWAKYSNFDVATHVPLIFYVPGRTASLPEAGEKLFPYLDPFDSASQLMEPGRQSMDLVELVSLFPTLAGLAGLQVPPRCPVPSFHVELCREGKNLLKHFRFRDLEEDPYLPGNPRELIAYSQYPRPSDIPQWNSDKPSLKDIKIMGYSIRTIDYRYTVWVGFNPDEFLANFSDIHAGELYFVDSDPLQDHNMYNDSQGGDLFQLLMP

SEQ ID NO: 59 - DNA, 15 bp, synthetic construct
  source 1..15: mol_type = other DNA
  misc_feature 1..15: note = Amino acid sequence of an exemplified linker 6
ggggsggggsggggs

SEQ ID NO: 60 - protein, 656 aa, synthetic construct
  REGION 1..656: note = Amino acid sequence of VHH6-GS3-hIDS
QVQLVESGGGLVQPGGSLRLSCAASGSIFDIYVMRWYRQAPGKGLEWVASIYAGGRNDYDNVVKGRFTISRDNSKNTLYLQMNSLRAEDTAVYFCNVLTYAGRPYWGQGTQVTVSSGGGGSGGGGSGGGGSSETQANSTTDALNVLLIIVDDLRPSLGCYGDKLVRSPNIDQLASHSLLFQNAFAQQAVCAPSRVSFLTGRRPDTTRLYDFNSYWRVHAGNFSTIPQYFKENGYVTMSVGKVFHPGISSNHTDDSPYSWSFPPYHPSSEKYENTKTCRGPDGELHANLLCPVDVLDVPEGTLPDKQSTEQAIQLLEKMKTSASPFFLAVGYHKPHIPFRYPKEFQKLYPLENITLAPDPEVPDGLPPVAYNPWMDIRQREDVQALNISVPYGPIPVDFQRKIRQSYFASVSYLDTQVGRLLSALDDLQLANSTIIAFTSDHGWALGEHGEWAKYSNFDVATHVPLIFYVPGRTASLPEAGEKLFPYLDPFDSASQLMEPGRQSMDLVELVSLFPTLAGLAGLQVPPRCPVPSFHVELCREGKNLLKHFRFRDLEEDPYLPGNPRELIAYSQYPRPSDIPQWNSDKPSLKDIKIMGYSIRTIDYRYTVWVGFNPDEFLANFSDIHAGELYFVDSDPLQDHNMYNDSQGGDLFQLLMP

SEQ ID NO: 61 - DNA, 1968 bp, synthetic construct
  source 1..1968: mol_type = other DNA
  misc_feature 1..1968: note = Nucleotide sequence of VHH6-GS3-hIDS
caagtgcagctggtcgagagcggaggaggactggtccagcccggcggctctctgagactgagctgtgccgccagcggcagcatcttcgacatctacgtgatgaggtggtacaggcaagcccccggcaagggactggagtgggtcgccagcatctacgccggcggaaggaatgactacgacaacgtggtgaagggaaggttcactatctctagggacaacagcaagaacactctctatctgcagatgaactctctgagggctgaggatacagccgtgtacttctgcaacgtgctgacttatgccggaaggccatactggggacaaggcactcaggtgacagtgagcagcggagggggtggctccggtggagggggctccggaggtggaggatcctccgaaacgcaggccaactcgaccacagatgctctgaacgttcttctcatcatcgtggatgacctgcgcccctccctgggctgttatggggataagctggtgaggtccccaaatattgaccaactggcatcccacagcctcctcttccagaatgcctttgcgcagcaagcagtgtgcgccccgagccgcgtttctttcctcactggcaggagacctgacaccacccgcctgtacgacttcaactcctactggagggtgcacgctggaaacttctccaccatcccccagtacttcaaggagaatggctatgtgaccatgtcggtgggaaaagtctttcaccctgggatatcttctaaccataccgatgattctccgtatagctggtcttttccaccttatcatccttcctctgagaagtatgaaaacactaagacatgtcgagggccagatggagaactccatgccaacctgctttgccctgtggatgtgctggatgttcccgagggcaccttgcctgacaaacagagcactgagcaagccatacagttgttggaaaagatgaaaacgtcagccagtcctttcttcctggccgttgggtatcataagccacacatccccttcagataccccaaggaatttcagaagttgtatcccttggagaacatcaccctggcccccgatcccgaggtccctgatggcctaccccctgtggcctacaacccctggatggacatcaggcaacgggaagacgtccaagccttaaacatcagtgtgccgtatggtccaattcctgtggactttcagcggaaaatccgccagagctactttgcctctgtgtcatatttggatacacaggtcggccgcctcttgagtgctttggacgatcttcagctggccaacagcaccatcattgcatttacctcggatcatgggtgggctctaggtgaacatggagaatgggccaaatacagcaattttgatgttgctacccatgttcccctgatattctatgttcctggaaggacggcttcacttccggaggcaggcgagaagcttttcccttacctcgacccttttgattccgcctcacagttgatggagccaggcaggcaatccatggaccttgtggaacttgtgtctctttttcccacgctggctggacttgcaggactgcaggttccacctcgctgccccgttccttcatttcacgttgagctgtgcagagaaggcaagaaccttctgaagcattttcgattccgtgacttggaagaagatccgtacctccctggtaatccccgtgaactgattgcctatagccagtatccccggccttcagacatccctcagtggaattctgacaagccgagtttaaaagatataaagatcatgggctattccatacgcaccatagactataggtatactgtgtgggttggcttcaatcctgatgaatttctagctaacttttctgacatccatgcaggggaactgtattttgtggattctgacccattgcaggatcacaatatgtataatgattcccaaggtggagaccttttccagttgttgatgcct

SEQ ID NO: 62 - protein, 656 aa, synthetic construct
  REGION 1..656: note = Amino acid sequence of VHH5-GS3-hIDS
QVQLVESGGGLVQPGGSLRLSCAASGSIFDIYVMRWYRQAPGKGLEWVASIYDGGRNDYDNVVKGRFTISRDNSKNTLYLQMNSLRAEDTAVYFCNVLTYAGRPYWGQGTQVTVSSGGGGSGGGGSGGGGSSETQANSTTDALNVLLIIVDDLRPSLGCYGDKLVRSPNIDQLASHSLLFQNAFAQQAVCAPSRVSFLTGRRPDTTRLYDFNSYWRVHAGNFSTIPQYFKENGYVTMSVGKVFHPGISSNHTDDSPYSWSFPPYHPSSEKYENTKTCRGPDGELHANLLCPVDVLDVPEGTLPDKQSTEQAIQLLEKMKTSASPFFLAVGYHKPHIPFRYPKEFQKLYPLENITLAPDPEVPDGLPPVAYNPWMDIRQREDVQALNISVPYGPIPVDFQRKIRQSYFASVSYLDTQVGRLLSALDDLQLANSTIIAFTSDHGWALGEHGEWAKYSNFDVATHVPLIFYVPGRTASLPEAGEKLFPYLDPFDSASQLMEPGRQSMDLVELVSLFPTLAGLAGLQVPPRCPVPSFHVELCREGKNLLKHFRFRDLEEDPYLPGNPRELIAYSQYPRPSDIPQWNSDKPSLKDIKIMGYSIRTIDYRYTVWVGFNPDEFLANFSDIHAGELYFVDSDPLQDHNMYNDSQGGDLFQLLMP

SEQ ID NO: 63 - DNA, 1968 bp, synthetic construct
  source 1..1968: mol_type = other DNA
  misc_feature 1..1968: note = Nucleotide sequence of VHH5-GS3-hIDS
caagtgcagctggtcgagagcggaggaggactggtccagcccggcggctctctgagactgagctgtgccgccagcggcagcatcttcgacatctacgtgatgaggtggtacaggcaagcccccggcaagggactggagtgggtcgccagcatctacgatggcggaaggaatgactacgacaacgtggtgaagggaaggttcactatctctagggacaacagcaagaacactctctatctgcagatgaactctctgagggctgaggatacagccgtgtacttctgcaacgtgctgacttatgccggaaggccatactggggacaaggcactcaggtgacagtgagcagcggtggcggagggtctggaggtggcggatcaggcggaggtggatcctccgaaacgcaggccaactcgaccacagatgctctgaacgttcttctcatcatcgtggatgacctgcgcccctccctgggctgttatggggataagctggtgaggtccccaaatattgaccaactggcatcccacagcctcctcttccagaatgcctttgcgcagcaagcagtgtgcgccccgagccgcgtttctttcctcactggcaggagacctgacaccacccgcctgtacgacttcaactcctactggagggtgcacgctggaaacttctccaccatcccccagtacttcaaggagaatggctatgtgaccatgtcggtgggaaaagtctttcaccctgggatatcttctaaccataccgatgattctccgtatagctggtcttttccaccttatcatccttcctctgagaagtatgaaaacactaagacatgtcgagggccagatggagaactccatgccaacctgctttgccctgtggatgtgctggatgttcccgagggcaccttgcctgacaaacagagcactgagcaagccatacagttgttggaaaagatgaaaacgtcagccagtcctttcttcctggccgttgggtatcataagccacacatccccttcagataccccaaggaatttcagaagttgtatcccttggagaacatcaccctggcccccgatcccgaggtccctgatggcctaccccctgtggcctacaacccctggatggacatcaggcaacgggaagacgtccaagccttaaacatcagtgtgccgtatggtccaattcctgtggactttcagcggaaaatccgccagagctactttgcctctgtgtcatatttggatacacaggtcggccgcctcttgagtgctttggacgatcttcagctggccaacagcaccatcattgcatttacctcggatcatgggtgggctctaggtgaacatggagaatgggccaaatacagcaattttgatgttgctacccatgttcccctgatattctatgttcctggaaggacggcttcacttccggaggcaggcgagaagcttttcccttacctcgacccttttgattccgcctcacagttgatggagccaggcaggcaatccatggaccttgtggaacttgtgtctctttttcccacgctggctggacttgcaggactgcaggttccacctcgctgccccgttccttcatttcacgttgagctgtgcagagaaggcaagaaccttctgaagcattttcgattccgtgacttggaagaagatccgtacctccctggtaatccccgtgaactgattgcctatagccagtatccccggccttcagacatccctcagtggaattctgacaagccgagtttaaaagatataaagatcatgggctattccatacgcaccatagactataggtatactgtgtgggttggcttcaatcctgatgaatttctagctaacttttctgacatccatgcaggggaactgtattttgtggattctgacccattgcaggatcacaatatgtataatgattcccaaggtggagaccttttccagttgttgatgcct

SEQ ID NO: 64 - protein, 774 aa, synthetic construct
  REGION 1..774: note = Amino acid sequence of VHH5-Tandem-GS3-hIDS
QVQLVESGGGLVQPGGSLRLSCAASGSIFDIYVMRWYRQAPGKGLEWVASIYDGGRNDYDNVVKGRFTISRDNSKNTLYLQMNSLRAEDTAVYFCNVLTYAGRPYWGQGTQVTVSSGSQVQLVESGGGLVQPGGSLRLSCAASGSIFDIYVMRWYRQAPGKGLEWVASIYDGGRNDYDNVVKGRFTISRDNSKNTLYLQMNSLRAEDTAVYFCNVLTYAGRPYWGQGTQVTVSSGGGGSGGGGSGGGGSSETQANSTTDALNVLLIIVDDLRPSLGCYGDKLVRSPNIDQLASHSLLFQNAFAQQAVCAPSRVSFLTGRRPDTTRLYDFNSYWRVHAGNFSTIPQYFKENGYVTMSVGKVFHPGISSNHTDDSPYSWSFPPYHPSSEKYENTKTCRGPDGELHANLLCPVDVLDVPEGTLPDKQSTEQAIQLLEKMKTSASPFFLAVGYHKPHIPFRYPKEFQKLYPLENITLAPDPEVPDGLPPVAYNPWMDIRQREDVQALNISVPYGPIPVDFQRKIRQSYFASVSYLDTQVGRLLSALDDLQLANSTIIAFTSDHGWALGEHGEWAKYSNFDVATHVPLIFYVPGRTASLPEAGEKLFPYLDPFDSASQLMEPGRQSMDLVELVSLFPTLAGLAGLQVPPRCPVPSFHVELCREGKNLLKHFRFRDLEEDPYLPGNPRELIAYSQYPRPSDIPQWNSDKPSLKDIKIMGYSIRTIDYRYTVWVGFNPDEFLANFSDIHAGELYFVDSDPLQDHNMYNDSQGGDLFQLLMP

SEQ ID NO: 65 - DNA, 2322 bp, synthetic construct
  source 1..2322: mol_type = other DNA
  misc_feature 1..2322: note = Nucleotide sequence of VHH5-Tandem-GS3-hIDS
caagtgcagctggtcgagagcggaggaggactggtccagcccggcggctctctgagactgagctgtgccgccagcggcagcatcttcgacatctacgtgatgaggtggtacaggcaagcccccggcaagggactggagtgggtcgccagcatctacgatggcggaaggaatgactacgacaacgtggtgaagggaaggttcactatctctagggacaacagcaagaacactctctatctgcagatgaactctctgagggctgaggatacagccgtgtacttctgcaacgtgctgacttatgccggaaggccatactggggacaaggcactcaggtgacagtgagcagcggatcccaagtgcagctggtcgagagcggaggaggactggtccagcccggcggctctctgagactgagctgtgccgccagcggcagcatcttcgacatctacgtgatgaggtggtacaggcaagcccccggcaagggactggagtgggtcgccagcatctacgatggcggaaggaatgactacgacaacgtggtgaagggaaggttcactatctctagggacaacagcaagaacactctctatctgcagatgaactctctgagggctgaggatacagccgtgtacttctgcaacgtgctgacttatgccggaaggccatactggggacaaggcactcaggtgacagtgagcagcggagggggtggctccggtggagggggctccggaggtggaggatcctccgaaacgcaggccaactcgaccacagatgctctgaacgttcttctcatcatcgtggatgacctgcgcccctccctgggctgttatggggataagctggtgaggtccccaaatattgaccaactggcatcccacagcctcctcttccagaatgcctttgcgcagcaagcagtgtgcgccccgagccgcgtttctttcctcactggcaggagacctgacaccacccgcctgtacgacttcaactcctactggagggtgcacgctggaaacttctccaccatcccccagtacttcaaggagaatggctatgtgaccatgtcggtgggaaaagtctttcaccctgggatatcttctaaccataccgatgattctccgtatagctggtcttttccaccttatcatccttcctctgagaagtatgaaaacactaagacatgtcgagggccagatggagaactccatgccaacctgctttgccctgtggatgtgctggatgttcccgagggcaccttgcctgacaaacagagcactgagcaagccatacagttgttggaaaagatgaaaacgtcagccagtcctttcttcctggccgttgggtatcataagccacacatccccttcagataccccaaggaatttcagaagttgtatcccttggagaacatcaccctggcccccgatcccgaggtccctgatggcctaccccctgtggcctacaacccctggatggacatcaggcaacgggaagacgtccaagccttaaacatcagtgtgccgtatggtccaattcctgtggactttcagcggaaaatccgccagagctactttgcctctgtgtcatatttggatacacaggtcggccgcctcttgagtgctttggacgatcttcagctggccaacagcaccatcattgcatttacctcggatcatgggtgggctctaggtgaacatggagaatgggccaaatacagcaattttgatgttgctacccatgttcccctgatattctatgttcctggaaggacggcttcacttccggaggcaggcgagaagcttttcccttacctcgacccttttgattccgcctcacagttgatggagccaggcaggcaatccatggaccttgtggaacttgtgtctctttttcccacgctggctggacttgcaggactgcaggttccacctcgctgccccgttccttcatttcacgttgagctgtgcagagaaggcaagaaccttctgaagcattttcgattccgtgacttggaagaagatccgtacctccctggtaatccccgtgaactgattgcctatagccagtatccccggccttcagacatccctcagtggaattctgacaagccgagtttaaaagatataaagatcatgggctattccatacgcaccatagactataggtatactgtgtgggttggcttcaatcctgatgaatttctagctaacttttctgacatccatgcaggggaactgtattttgtggattctgacccattgcaggatcacaatatgtataatgattcccaaggtggagaccttttccagttgttgatgcct

SEQ ID NO: 66 - protein, 482 aa, Homo sapiens
  REGION 1..482: note = Amino acid sequence of hSGSH
RPRNALLLLADDGGFESGAYNNSAIATPHLDALARRSLLFRNAFTSVSSCSPSRASLLTGLPQHQNGMYGLHQDVHHFNSFDKVRSLPLLLSQAGVRTGIIGKKHVGPETVYPFDFAYTEENGSVLQVGRNITRIKLLVRKFLQTQDDRPFFLYVAFHDPHRCGHSQPQYGTFCEKFGNGESGMGRIPDWTPQAYDPLDVLVPYFVPNTPAARADLAAQYTTVGRMDQGVGLVLQELRDAGVLNDTLVIFTSDNGIPFPSGRTNLYWPGTAEPLLVSSPEHPKRWGQVSEAYVSLLDLTPTILDWFSIPYPSYAIFGSKTIHLTGRSLLPALEAEPLWATVFGSQSHHEVTMSYPMRSVQHRHFRLVHNLNFKMPFPIDQDFYVSPTFQDLLNRTTAGQPTGWYKDLRHYYYRARWELYDRSRDPHETQNLATDPRFAQLLEMLRDQLAKWQWETHDPWVCAPDGVLEEKLSPQCQPLHNEL

SEQ ID NO: 67 - protein, 621 aa, synthetic construct
  REGION 1..621: note = Amino acid sequence of VHH3-GS3-hSGSH
DYKDDDDKQVQLVESGGGLVQPGESLRLSCAASGSIFDIYVMRWYRQAPGNQREWVASIYDGGRNDYDNVVKGRFTISRDNAKNTVHLQMNSLKPEDTAVYFCNVLTYAGRPYWGQGTQVTVSSGGGGSGGGGSGGGGSRPRNALLLLADDGGFESGAYNNSAIATPHLDALARRSLLFRNAFTSVSSCSPSRASLLTGLPQHQNGMYGLHQDVHHFNSFDKVRSLPLLLSQAGVRTGIIGKKHVGPETVYPFDFAYTEENGSVLQVGRNITRIKLLVRKFLQTQDDRPFFLYVAFHDPHRCGHSQPQYGTFCEKFGNGESGMGRIPDWTPQAYDPLDVLVPYFVPNTPAARADLAAQYTTVGRMDQGVGLVLQELRDAGVLNDTLVIFTSDNGIPFPSGRTNLYWPGTAEPLLVSSPEHPKRWGQVSEAYVSLLDLTPTILDWFSIPYPSYAIFGSKTIHLTGRSLLPALEAEPLWATVFGSQSHHEVTMSYPMRSVQHRHFRLVHNLNFKMPFPIDQDFYVSPTFQDLLNRTTAGQPTGWYKDLRHYYYRARWELYDRSRDPHETQNLATDPRFAQLLEMLRDQLAKWQWETHDPWVCAPDGVLEEKLSPQCQPLHNEL

SEQ ID NO: 68 - DNA, 1863 bp, synthetic construct
  source 1..1863: mol_type = other DNA
  misc_feature 1..1863: note = Nucleotide sequence of VHH3-GS3-hSGSH
gactacaaagacgatgacgacaagcaggtgcagctcgtggagtctgggggaggcttggtacagcctggggaatctctgagactctcctgtgcagcctctggaagcatcttcgatatctatgtcatgcgctggtaccgccaggctccagggaaccagcgcgaatgggtcgcaagtatttatgatggcggtaggaacgactatgataatgtcgtgaagggccgattcaccatctccagagacaacgccaagaacacggtgcatctgcaaatgaacagcctgaaacccgaagatacggccgtctatttttgtaatgtgctaacatacgcaggccgtccctactggggccaggggacccaggtcaccgtctcctcaggtggcggagggtctggaggtggcggatcaggcggaggtggatcccgtccccggaacgcactgctgctcctcgcggatgacggaggctttgagagtggcgcgtacaacaacagcgccatcgccaccccgcacctggacgccttggcccgccgcagcctcctctttcgcaatgccttcacctcggtcagcagctgctctcccagccgcgccagcctcctcactggcctgccccagcatcagaatgggatgtacgggctgcaccaggacgtgcaccacttcaactccttcgacaaggtgcggagcctgccgctgctgctcagccaagctggtgtgcgcacaggcatcatcgggaagaagcacgtggggccggagaccgtgtacccgtttgactttgcgtacacggaggagaatggctccgtcctccaggtggggcggaacatcactagaattaagctgctcgtccggaaattcctgcagactcaggatgaccggcctttcttcctctacgtcgccttccacgacccccaccgctgtgggcactcccagccccagtacggaaccttctgtgagaagtttggcaacggagagagcggcatgggtcgtatcccagactggaccccccaggcctacgacccactggacgtgctggtgccttacttcgtccccaacaccccggcagcccgagccgacctggccgctcagtacaccaccgtcggccgcatggaccaaggagttggactggtgctccaggagctgcgtgacgccggtgtcctgaacgacacactggtgatcttcacgtccgacaacggtatccccttccccagcggcaggaccaacctgtactggccgggcactgctgaacccttactggtgtcatccccggagcacccaaaacgctggggccaagtcagcgaggcctacgtgagcctcctagacctcacgcccaccatcttggattggttctcgatcccgtaccccagctacgccatctttggctcgaagaccatccacctcactggccggtccctcctgccggcgctggaggccgagcccctctgggccaccgtctttggcagccagagccaccacgaggtcaccatgtcctaccccatgcgctccgtgcagcaccggcacttccgcctcgtgcacaacctcaacttcaagatgccctttcccatcgaccaggacttctacgtctcacccaccttccaggacctcctgaaccgcaccacagctggtcagcccacgggctggtacaaggacctccgtcattactactaccgggcgcgctgggagctctacgaccggagccgggacccccacgagacccagaacctggccaccgacccgcgctttgctcagcttctggagatgcttcgggaccagctggccaagtggcagtgggagacccacgacccctgggtgtgcgcccccgacggcgtcctggaggagaagctctctccccagtgccagcccctccacaatgagctg

SEQ ID NO: 69 - protein, 28 aa, synthetic construct
  REGION 1..28: note = Amino acid sequence of an exemplified linker 7
GGGGSGGGGSGGGGSGGGGSGGGGSGGS